European Patent Application EP 4 458 419 A2, published November 6, 2024. Title: METHODS FOR EXPANDING ANTIGEN-SPECIFIC CAR-T CELLS, COMPOSITIONS AND USES RELATED THERETO. Applicant: Atara Biotherapeutics, Inc. The sequence listing filed with the application follows.

SEQUENCE LISTING (26 sequences)

SEQ ID NO: 1 - protein, 376 aa, Human gammaherpesvirus 4
MDLDLERGPPGPRRPPRGPPLSSYIALALLLLLLALLFWLYIIMSNWTGGALLVLYAFALMLVIIILIIFIFRRDLLCPLGALCLLLLMITLLLIALWNLHGQALYLGIVLFIFGCLLVLGIWVYFLEILWRLGATIWQLLAFFLAFFLDILLLIIALYLQQNWWTLLVDLLWLLLFLAILIWMYYHGQRHSDEHHHDDSLPHPQQATDDSSNHSDSNSNEGRHHLLVSGAGDAPPLCSQNLGAPGGGPDNGPQDPDNTDDNGPQDPDNTDDNGPHDPLPQDPDNTDDNGPQDPDNTDDNGPHDPLPHNPSDSAGNDGGPPNLTEEVENKGGDRGPPSMTDGGGGDPHLPTLLLGTSGSGGDDDDPHGPVQLSYYD

SEQ ID NO: 2 - protein, 497 aa, Human gammaherpesvirus 4
MGSLEMVPMGAGPPSPGGDPDGDDGGNNSQYPSASGSDGNTPTPPNDEERESNEEPPPPYEDLDWGNGDRHSDYQPLGNQDPSLYLGLQHDGNDGLPPPPYSPRDDSSQHIYEEAGRGSMNPVCLPVIVAPYLFWLAAIAASCFTASVSTVVTATGLALSLLLLAAVASSYAAAQRKLLTPVTVLTAVVTFFAICLTWRIEDPPFNSLLFALLAAAGGLQGIYVLVMLVLLILAYRRRWRRLTVCGGIMFLACVLVLIVDAVLQLSPLLGAVTVVSMTLLLLAFVLWLSSPGGLGTLGAALLTLAAALALLASLILGTLNLTTMFLLMLLWTLVVLLICSSCSSCPLTKILLARLFLYALALLLLASALIAGGSILQTNFKSLSSTEFIPNLFCMLLLIVAGILFILAILTEWGSGNRTYGPVFMCLGGLLTMVAGAVWLTVMTNTLLSAWILTAGFLIFLIGFALFGVIRCCRYCCYYCLTLESEERPPTPYRNTV

SEQ ID NO: 3 - protein, 238 aa, Human gammaherpesvirus 4
PFFHPVGEADYFEYLQEGGPDGEPDVPPGAIEQGPADDPGEGPSTGPRGQGDGGRRKKGGWFGKHRGQGGSNPKFENIAEGLRVLLARSHVERTTEEGTWVAGVFVYGGSKTSLYNLRRGTALAIPQCRLTPLSRLPFGMAPGPGPQPGPLRESIVCYFMVFLQTHIFAEVLKDAIKDLVMTKPAPTCNIKVTVCSFDDGVDLPPWFPPMVEGAAAEGDDGDDGDEGGDGDEGEEGQE

SEQ ID NO: 4 - protein, 9 aa, Human gammaherpesvirus 4
CLGGLLTMV

SEQ ID NO: 5 - protein, 9 aa, Human gammaherpesvirus 4
FLYALALLL

SEQ ID NO: 6 - protein, 9 aa, Human gammaherpesvirus 4
YLQQNWWTL

SEQ ID NO: 7 - protein, 9 aa, Human gammaherpesvirus 4
YLLEMLWRL

SEQ ID NO: 8 - protein, 9 aa, Human gammaherpesvirus 4
ALLVLYSFA

SEQ ID NO: 9 - protein, 9 aa, Human gammaherpesvirus 4
LLSAWILTA

SEQ ID NO: 10 - protein, 9 aa, Human gammaherpesvirus 4
LTAGFLIFL

SEQ ID NO: 11 - protein, 11 aa, Human gammaherpesvirus 4
SSCSSCPLSKI

SEQ ID NO: 12 - protein, 8 aa, Human gammaherpesvirus 4
PYLFWLAA

SEQ ID NO: 13 - protein, 9 aa, Human gammaherpesvirus 4
TYGPVFMCL

SEQ ID NO: 14 - protein, 10 aa, Human gammaherpesvirus 4
VMSNTLLSAW

SEQ ID NO: 15 - protein, 8 aa, Human gammaherpesvirus 4
CPLSKILL

SEQ ID NO: 16 - protein, 9 aa, Human gammaherpesvirus 4
RRRWRRLTV

SEQ ID NO: 17 - protein, 9 aa, Human gammaherpesvirus 4
IEDPPFNSL

SEQ ID NO: 18 - protein, 9 aa, Human gammaherpesvirus 4
IALYLQQNW

SEQ ID NO: 19 - protein, 9 aa, Human gammaherpesvirus 4
MSNTLLSAW

SEQ ID NO: 20 - protein, 9 aa, Human gammaherpesvirus 4
VLKDAIKDL

SEQ ID NO: 21 - protein, 9 aa, Human gammaherpesvirus 4
RPQKRPSCI

SEQ ID NO: 22 - protein, 9 aa, Human gammaherpesvirus 4
IPQCRLTPL

SEQ ID NO: 23 - protein, 9 aa, Human gammaherpesvirus 4
YNLRRGTAL

SEQ ID NO: 24 - protein, 11 aa, Human gammaherpesvirus 4
HPVGEADYFEY

SEQ ID NO: 25 - protein, 9 aa, Human gammaherpesvirus 4
LSRLPFGMA

SEQ ID NO: 26 - protein, 10 aa, Human gammaherpesvirus 4
FVYGGSKTSL